European Patent Specification EP 4 019 639 B1, published June 24, 2026. Title: PROMOTING REGENERATION AND TRANSFORMATION IN PLANTS. Applicant: KWS SAAT SE & Co. KGaA. The sequence listing filed with the application follows.

SEQUENCE LISTING (17 sequences)

SEQ ID NO: 1 - DNA, 1737 bp, Artificial Sequence
  cDNA of Brassica napus Babyboom
atggataataactggttaggcttttctctctctccttatgaacaaaatcaccatcgtaaggacgtctactcttccaccaccacaaccgtcgtagatgtcgccggagagtactgttacgatccgaccgctgcctccgatgagtcttcagccatccaaacatcgtttccttctccctttggtgtcgtcgtcgatgctttcaccagagacaacaatagtcactcccgagattgggacatcaatggttgtgcatgcaataacatccacaacgatgagcaagatggaccaaagcttgagaatttccttggccgcaccaccacgatttacaacaccaacgaaaacgttggagatggaagtggaagtggctgttatggaggaggagacggtggtggtggctcactaggactttcgatgataaagacatggctgagaaatcaacccgtggataatgttgataatcaagaaaatggcaatgctgcaaaaggcctgtccctctcaatgaactcatctacttcttgtgataacaacaacgacagcaataacaacgttgttgcccaagggaagactattgatgatagcgttgaagctacaccgaagaaaactattgagagttttggacagaggacgtctatataccgcggtgttacaaggcatcggtggacaggaagatatgaggcacatttatgggataatagttgtaaaagagaaggccaaacgcgcaaaggaagacaagtttatttgggaggttatgacaaagaagaaaaagcagctagggcttatgatttagccgcactcaagtattggggaaccaccactactactaacttccccatgagcgaatatgaaaaagaggtagaagagatgaagcacatgacaaggcaagagtatgttgcctcactgcgcaggaaaagtagtggtttctctcgtggtgcatcgatttatcgtggagtaacaagacatcaccaacatggaagatggcaagctaggataggaagagtcgccggtaacaaagacctctacttgggaacttttggcacacaagaagaagctgcagaggcatacgacattgcggccatcaaattcagaggattaaccgcagtgactaacttcgacatgaacagatacaacgttaaagcaatcctcgaaagccctagtcttcctattggtagcgccgcaaaacgtctcaaggaggctaaccgtccggttccaagtatgatgatgatcagtaataacgtttcagagagtgagaatagtgctagcggttggcaaaacgctgcggttcagcatcatcagggagtagatttgagcttattgcaccaacatcaagagaggtacaatggttattattacaatggaggaaacttgtcttcggagagtgctagggcttgtttcaaacaagaggatgatcaacaccatttcttgagcaacacgcagagcctcatgactaatatcgatcatcaaagttctgtttcggatgattcggttactgtttgtggaaatgttgttggttatggtggttatcaaggatttgcagccccggttaactgcgatgcctacgctgctagtgagtttgattataacgcaagaaaccattattactttgctcagcagcagcagacccagcagtcgccaggtggagattttcccgcggcaatgacgaataatgttggctctaatatgtattaccatggggaaggtggtggagaagttgctccaacatttacagtttggaacgacaat

SEQ ID NO: 2 - protein, 579 aa, Brassica napus
MDNNWLGFSLSPYEQNHHRKDVYSSTTTTVVDVAGEYCYDPTAASDESSAIQTSFPSPFGVVVDAFTRDNNSHSRDWDINGCACNNIHNDEQDGPKLENFLGRTTTIYNTNENVGDGSGSGCYGGGDGGGGSLGLSMIKTWLRNQPVDNVDNQENGNAAKGLSLSMNSSTSCDNNNDSNNNVVAQGKTIDDSVEATPKKTIESFGQRTSIYRGVTRHRWTGRYEAHLWDNSCKREGQTRKGRQVYLGGYDKEEKAARAYDLAALKYWGTTTTTNFPMSEYEKEVEEMKHMTRQEYVASLRRKSSGFSRGASIYRGVTRHHQHGRWQARIGRVAGNKDLYLGTFGTQEEAAEAYDIAAIKFRGLTAVTNFDMNRYNVKAILESPSLPIGSAAKRLKEANRPVPSMMMISNNVSESENSASGWQNAAVQHHQGVDLSLLHQHQERYNGYYYNGGNLSSESARACFKQEDDQHHFLSNTQSLMTNIDHQSSVSDDSVTVCGNVVGYGGYQGFAAPVNCDAYAASEFDYNARNHYYFAQQQQTQQSPGGDFPAAMTNNVGSNMYYHGEGGGEVAPTFTVWNDN

SEQ ID NO: 3 - DNA, 1974 bp, Artificial Sequence
  cDNA sequence of Brassica napus Babyboom with 3 UTR
atggataataactggttaggcttttctctctctccttatgaacaaaatcaccatcgtaaggacgtctactcttccaccaccacaaccgtcgtagatgtcgccggagagtactgttacgatccgaccgctgcctccgatgagtcttcagccatccaaacatcgtttccttctccctttggtgtcgtcgtcgatgctttcaccagagacaacaatagtcactcccgagattgggacatcaatggttgtgcatgcaataacatccacaacgatgagcaagatggaccaaagcttgagaatttccttggccgcaccaccacgatttacaacaccaacgaaaacgttggagatggaagtggaagtggctgttatggaggaggagacggtggtggtggctcactaggactttcgatgataaagacatggctgagaaatcaacccgtggataatgttgataatcaagaaaatggcaatgctgcaaaaggcctgtccctctcaatgaactcatctacttcttgtgataacaacaacgacagcaataacaacgttgttgcccaagggaagactattgatgatagcgttgaagctacaccgaagaaaactattgagagttttggacagaggacgtctatataccgcggtgttacaaggcatcggtggacaggaagatatgaggcacatttatgggataatagttgtaaaagagaaggccaaacgcgcaaaggaagacaagtttatttgggaggttatgacaaagaagaaaaagcagctagggcttatgatttagccgcactcaagtattggggaaccaccactactactaacttccccatgagcgaatatgaaaaagaggtagaagagatgaagcacatgacaaggcaagagtatgttgcctcactgcgcaggaaaagtagtggtttctctcgtggtgcatcgatttatcgtggagtaacaagacatcaccaacatggaagatggcaagctaggataggaagagtcgccggtaacaaagacctctacttgggaacttttggcacacaagaagaagctgcagaggcatacgacattgcggccatcaaattcagaggattaaccgcagtgactaacttcgacatgaacagatacaacgttaaagcaatcctcgaaagccctagtcttcctattggtagcgccgcaaaacgtctcaaggaggctaaccgtccggttccaagtatgatgatgatcagtaataacgtttcagagagtgagaatagtgctagcggttggcaaaacgctgcggttcagcatcatcagggagtagatttgagcttattgcaccaacatcaagagaggtacaatggttattattacaatggaggaaacttgtcttcggagagtgctagggcttgtttcaaacaagaggatgatcaacaccatttcttgagcaacacgcagagcctcatgactaatatcgatcatcaaagttctgtttcggatgattcggttactgtttgtggaaatgttgttggttatggtggttatcaaggatttgcagccccggttaactgcgatgcctacgctgctagtgagtttgattataacgcaagaaaccattattactttgctcagcagcagcagacccagcagtcgccaggtggagattttcccgcggcaatgacgaataatgttggctctaatatgtattaccatggggaaggtggtggagaagttgctccaacatttacagtttggaacgacaattagaaaaaatagttaaagatctttagttatatgcgttgttgtgtgctggtgaacagtgtgatactttgattatgtttttttctttctctttttctttttcttggttaatttcttaagacttatttttagtttccattagttggataaattttcagactaaaaaaaaaaaaaaaaaaaaactcgagggggggcccggtaccgagctcgaatttccccgatcgttcaaacatttgtacc

SEQ ID NO: 4 - DNA, 2603 bp, Artificial Sequence
  DNA sequence of Brassica napus Babyboom with rat glucocorticoid receptor domain
atggataataactggttaggcttttctctctctccttatgaacaaaatcaccatcgtaaggacgtctactcttccaccaccacaaccgtcgtagatgtcgccggagagtactgttacgatccgaccgctgcctccgatgagtcttcagccatccaaacatcgtttccttctccctttggtgtcgtcgtcgatgctttcaccagagacaacaatagtcactcccgagattgggacatcaatggttgtgcatgcaataacatccacaacgatgagcaagatggaccaaagcttgagaatttccttggccgcaccaccacgatttacaacaccaacgaaaacgttggagatggaagtggaagtggctgttatggaggaggagacggtggtggtggctcactaggactttcgatgataaagacatggctgagaaatcaacccgtggataatgttgataatcaagaaaatggcaatgctgcaaaaggcctgtccctctcaatgaactcatctacttcttgtgataacaacaacgacagcaataacaacgttgttgcccaagggaagactattgatgatagcgttgaagctacaccgaagaaaactattgagagttttggacagaggacgtctatataccgcggtgttacaaggcatcggtggacaggaagatatgaggcacatttatgggataatagttgtaaaagagaaggccaaacgcgcaaaggaagacaagtttatttgggaggttatgacaaagaagaaaaagcagctagggcttatgatttagccgcactcaagtattggggaaccaccactactactaacttccccatgagcgaatatgaaaaagaggtagaagagatgaagcacatgacaaggcaagagtatgttgcctcactgcgcaggaaaagtagtggtttctctcgtggtgcatcgatttatcgtggagtaacaagacatcaccaacatggaagatggcaagctaggataggaagagtcgccggtaacaaagacctctacttgggaacttttggcacacaagaagaagctgcagaggcatacgacattgcggccatcaaattcagaggattaaccgcagtgactaacttcgacatgaacagatacaacgttaaagcaatcctcgaaagccctagtcttcctattggtagcgccgcaaaacgtctcaaggaggctaaccgtccggttccaagtatgatgatgatcagtaataacgtttcagagagtgagaatagtgctagcggttggcaaaacgctgcggttcagcatcatcagggagtagatttgagcttattgcaccaacatcaagagaggtacaatggttattattacaatggaggaaacttgtcttcggagagtgctagggcttgtttcaaacaagaggatgatcaacaccatttcttgagcaacacgcagagcctcatgactaatatcgatcatcaaagttctgtttcggatgattcggttactgtttgtggaaatgttgttggttatggtggttatcaaggatttgcagccccggttaactgcgatgcctacgctgctagtgagtttgattataacgcaagaaaccattattactttgctcagcagcagcagacccagcagtcgccaggtggagattttcccgcggcaatgacgaataatgttggctctaatatgtattaccatggggaaggtggtggagaagttgctccaacatttacagtttggaacgacaatggatctacaaagaaaaaaatcaaagggattcagcaagccactgcaggagtctcacaagacacttcggaaaatcctaacaaaacaatagttcctgctgcattaccacagctcacccctaccttggtgtcactgctggaggtgattgaacccgaggtgttgtatgcaggatatgatagctctgttccagattcagcgtggagaattatgaccacactcaacatgttaggtgggcgtcaagtgattgcagcagtgaaatgggcaaaggcgataccaggcttcagaaacttacacctggatgaccaaatgaccctgctacagtactcatggatgtttctcatggcatttgccctgggttggagatcatacagacaatcaagtggaaacctgctctgctttgctcctgatctgattattaatgagcagagaatgtctctaccctgcatgtatgaccaatgtaaacacatgctgtttgtctcctctgaattacaaagattgcaggtatcctatgaagagtatctctgtatgaaaaccttactgcttctctcctcagttcctaaggaaggtctgaagagccaagagttatttgatgagattcgaatgacttatatcaaagagctaggaaaagccatcgtcaaaagggaagggaactccagtcagaactggcaacggttttaccaactgacaaagcttctggactccatgcatgaggtggttgagaatctccttacctactgcttccagacatttttggataagaccatgagtattgagttcccagagatgttagctgaaatcatcactaatcagataccaaaatattcaaatggaaatatcaaaaagctcctgtttcatcaaaaatgacaccc

SEQ ID NO: 5 - DNA, 11632 bp, Artificial Sequence
  vector pZFNnptII
cggccgcgtcgagcgatctagtaacatagatgacaccgcgcgcgataatttatcctagtttgcgcgctatattttgttttctatcgcgtattaaatgtataattgcgggactctaatcataaaaacccatctcataaataacgtcatgcattacatgttaattattacatgcttaacgtaattcaacagaaattatatgataatcatcgcaagaccggcaacaggattcaatcttaagaaactttattgccaaatgtttgaacgatcggggaaattcgagtcgagtttttcagcaagattctagacttgtacagctcgtccatgccgtacaggaacaggtggtggcggccctcggagcgctcgtactgttccacgatggtgtagtcctcgttgtgggaggtgatgtccagcttggtgtccacgtagtagtagccgggcagttgcacgggcttcttggccatgtagatggtcttgaactccaccaggtagtggccgccgtccttcagcttcagggcctggtggatctcgcccttcagcacgccgtcgcgggggtacaggcgctcggtggaggcctcccagcccatggtcttcttctgcattacggggccgtcgggggggaagttggtgccgcgcatcttcaccttgtagatcagcgtgccgtcctgcagggaggagtcctgggtcacggtcaccagaccgccgtcctcgaagttcatcacgcgctcccacttgaagccctcggggaaggacagcttcttgtaatcggggatgtcggcggggtgcttcacgtacgccttggagccgtacatgaactggggggacaggatgtcccaggcgaagggcagggggccgcccttggtcaccttcagcttggcggtctgggtgccctcgtaggggcggccctcgccctcgccctcgatctcgaactcgtggccgttcatggagccctccatgcgcaccttgaagcgcatgaactctttgatgacctcctcgcccttgctcaccatggtggcgggatcgcgccctatcgttcgtaaatggtgaaaattttcagaaaattgcttttgctttaaaagaaatgatttaaattgctgcaatagaagtagaatgcttgattgcttgagattcgtttgttttgtatatgttgtgttgagaggatccactagttctagagcggccgccaccgcggtggagctcgaattctcgaggtcctctccaaatgaaatgaacttccttatatagaggaagggtcttgcgaaggatagtgggattgtgcgtcatcccttacgtcagtggagatatcacatcaatccacttgctttgaagacgtggttggaacgtcttctttttccacgatgttcctcgtgggtgggggtccatctttgggaccactgtcggtagaggcatcttgaacgatagcctttcctttatcgcaatgatggcatttgtagaagccatcttccttttctactgtcctttcgatgaagtgacagatagctgggcaatggaatccgaggaggtttcccgatattaccctttgttgaaaagtctcaatagccctctggtcttctgagactgtatctttgatattcttggagtagacgagagtgtcgtgctccaccatgtatcacatcaatccacttgctttgaagacgtggttggaacgtcttctttttccacgatgttcctcgtgggtgggggtccatctttgggaccactgtcggtagaggcatcttgaacgatagcctttcctttatcgcaatgatggcatttgtagaagccatcttccttttctactgtcctttcgatgaagtgacagatagctgggcaatggaatccgaggaggtttcccgatattaccctttgttgaaaagtctcaatagccctctggtcttctgaacctgcaggcatgcaagctctagtaaggccttaagggccagatcttgggcccggtacccgatcagattgtcgtttcccgccttcggtttaaactatcagtgtttgacaggatatattggcgggtaaacctaagagaaaagagcgtttattagaataatcggatatttaaaagggcgtgaaaaggtttatccgttcgtccatttgtatgtgcatgccaaccacagggttcccctcgggagtgcttggcattccgtgcgataatgacttctgttcaaccacccaaacgtcggaaagcctgacgacggagcagcattccaaaaagatcccttggctcgtctgggtcggctagaaggtcgagtgggctgctgtggcttgatccctcaacgcggtcgcggacgtagcgcagcgccgaaaaatcctcgatcgcaaatccgacgctgtcgaaaagcgtgatctgcttgtcgctctttcggccgacgtcctggccagtcatcacgcgccaaagttccgtcacaggatgatctggcgcgagttgctggatctcgccttcaatccgggtctgtggcgggaactccacgaaaatatccgaacgcagcaagatatcgcggtgcatctcggtcttgcctgggcagtcgccgccgacgccgttgatgtggacgccgaaaaggatctaggtgaagatcctttttgataatctcatgaccaaaatcccttaacgtgagttttcgttccactgagcgtcagaccccgtagaaaagatcaaaggatcttcttgagatcctttttttctgcgcgtaatctgctgcttgcaaacaaaaaaaccaccgctaccagcggtggtttgtttgccggatcaagagctaccaactctttttccgaaggtaactggcttcagcagagcgcagataccaaatactgttcttctagtgtagccgtagttaggccaccacttcaagaactctgtagcaccgcctacatacctcgctctgctaatcctgttaccagtggctgctgccagtggcgataagtcgtgtcttaccgggttggactcaagacgatagttaccggataaggcgcagcggtcgggctgaacggggggttcgtgcacacagcccagcttggagcgaacgacctacaccgaactgagatacctacagcgtgagctatgagaaagcgccacgcttcccgaagggagaaaggcggacaggtatccggtaagcggcagggtcggaacaggagagcgcacgagggagcttccagggggaaacgcctggtatctttatagtcctgtcgggtttcgccacctctgacttgagcgtcgatttttgtgatgctcgtcaggggggcggagcctatggaaaaacgccagcaacgcggcctttttacggttcctggccttttgctggccttttgctcacatgttctttcctgcgttatcccctgattctgtggataaccgattaccgcctttgagtgagctgataccgctcgccgcagccgaacgaccgagcgcagcgagtcagtgagcgaggaagcggaagagcgcctgatgcggtattttctccttacgcatctgtgcggtatttcacaccgcatatggtgcactctcagtacaatctgctctgatgccgcatagttaagccagtatacactccgctatcgctacgtgactgggtcatggctgcgccccgacacccgccaacacccgctgacgcgccctgacgggcttgtctgctcccggcatccgcttacagacaagctgtgaccgtctccgggagctgcatgtgtcagaggttttcaccgtcatcaccgaaacgcgcgaggcaggggtacgtcgaggtcgatccaacccctccgctgctatagtgcagtcggcttctgacgttcagtgcagccgtcttctgaaaacgacatgtcgcacaagtcctaagttacgcgacaggctgccgccctgcccttttcctggcgttttcttgtcgcgtgttttagtcgcataaagtagaatacttgcgactagaaccggagacattacgccatgaacaagagcgccgccgctggcctgctgggctatgcccgcgtcagcaccgacgaccaggacttgaccaaccaacgggccgaactgcacgcggccggctgcaccaagctgttttccgagaagatcaccggcaccaggcgcgaccgcccggagctggccaggatgcttgaccacctacgccctggcgacgttgtgacagtgaccaggctagaccgcctggcccgcagcacccgcgacctactggacattgccgagcgcatccaggaggccggcgcgggcctgcgtagcctggcagagccgtgggccgacaccaccacgccggccggccgcatggtgttgaccgtgttcgccggcattgccgagttcgagcgttccctaatcatcgaccgcacccggagcgggcgcgaggccgccaaggcgcgaggcgtgaagtttggcccccgccctaccctcaccccggcacagatcgcgcacgcccgcgagctgatcgaccaggaaggccgcaccgtgaaagaggcggctgcactgcttggcgtgcatcgctcgaccctgtaccgcgcacttgagcgcagcgaggaagtgacgcccaccgaggccaggcggcgcggtgccttccgtgaggacgcattgaccgaggccgacgccctggcggccgccgagaatgaacgccaagaggaacaagcatgaaaccgcaccaggacggccaggacgaaccgtttttcattaccgaagagatcgaggcggagatgatcgcggccgggtacgtgttcgagccgcccgcgcacgtctcaaccgtgcggctgcatgaaatcctggccggtttgtctgatgccaagctcgcggcctggccggcgagcttggccgctgaagaaaccgagcgccgccgtctaaaaaggtgatgtgtatttgagtaaaacagcttgcgtcatgcggtcgctgcgtatatgatgcgatgagtaaataaacaaatacgcaaggggaacgcatgaaggttatcgctgtacttaaccagaaaggcgggtcaggcaagacgaccatcgcaacccatctagcccgcgccctgcaactcgccggggccgatgttctgttagtcgattccgatccccagggcagtgcccgcgattgggcggccgtgcgggaagatcaaccgctaaccgttgtcggcatcgaccgcccgacgattgaccgcgacgtgaaggccatcggccggcgcgacttcgtagtgatcgacggagcgccccaggcggcggacttggctgtgtccgcgatcaaggcagccgacttcgtgctgattccggtgcagccaagcccttacgacatatgggccaccgccgacctggtggagctggttaagcagcgcattgaggtcacggatggaaggctacaagcggcctttgtcgtgtcgcgggcgatcaaaggcacgcgcatcggcggtgaggttgccgaggcgctggccgggtacgagctgcccattcttgagtcccgtatcacgcagcgcgtgagctacccaggcactgccgccgccggcacaaccgttcttgaatcagaacccgagggcgacgctgcccgcgaggtccaggcgctggccgctgaaattaaatcaaaactcatttgagttaatgaggtaaagagaaaatgagcaaaagcacaaacacgctaagtgccggccgtccgagcgcacgcagcagcaaggctgcaacgttggccagcctggcagacacgccagccatgaagcgggtcaactttcagttgccggcggaggatcacaccaagctgaagatgtacgcggtacgccaaggcaagaccattaccgagctgctatctgaatacatcgcgcagctaccagagtaaatgagcaaatgaataaatgagtagatgaattttagcggctaaaggaggcggcatggaaaatcaagaacaaccaggcaccgacgccgtggaatgccccatgtgtggaggaacgggcggttggccaggcgtaagcggctgggttgtctgccggccctgcaatggcactggaacccccaagcccgaggaatcggcgtgagcggtcgcaaaccatccggcccggtacaaatcggcgcggcgctgggtgatgacctggtggagaagttgaaggcggcgcaggccgcccagcggcaacgcatcgaggcagaagcacgccccggtgaatcgtggcaagcggccgctgatcgaatccgcaaagaatcccggcaaccgccggcagccggtgcgccgtcgattaggaagccgcccaagggcgacgagcaaccagattttttcgttccgatgctctatgacgtgggcacccgcgatagtcgcagcatcatggacgtggccgttttccgtctgtcgaagcgtgaccgacgagctggcgaggtgatccgctacgagcttccagacgggcacgtagaggtttccgcagggccggccggcatggcgagtgtgtgggattacgacctggtactgatggcggtttcccatctaaccgaatccatgaaccgataccgggaagggaagggagacaagcccggccgcgtgttccgtccacacgttgcggacgtactcaagttctgccggcgagccgatggcggaaagcagaaagacgacctggtagaaacctgcattcggttaaacaccacgcacgttgccatgcagcgtacgaagaaggccaagaacggccgcctggtgacggtatccgagggtgaagccttgattagccgctacaagatcgtaaagagcgaaaccgggcggccggagtacatcgagatcgagctagctgattggatgtaccgcgagatcacagaaggcaagaacccggacgtgctgacggttcaccccgattactttttgatcgatcccggcatcggccgttttctctaccgcctggcacgccgcgccgcaggcaaggcagaagccagatggttgttcaagacgatctacgaacgcagtggcagcgccggagagttcaagaagttctgtttcaccgtgcgcaagctgatcgggtcaaatgacctgccggagtacgatttgaaggaggaggcggggcaggctggcccgatcctagtcatgcgctaccgcaacctgatcgagggcgaagcatccgccggttcctaatgtacggagcagatgctagggcaaattgccctagcaggggaaaaaggtcgaaaaggtctctttcctgtggatagcacgtacattgggaacccaaagccgtacattgggaaccggaacccgtacattgggaacccaaagccgtacattgggaaccggtcacacatgtaagtgactgatataaaagagaaaaaaggcgatttttccgcctaaaactctttaaaacttattaaaactcttaaaacccgcctggcctgtgcataactgtctggccagcgcacagccgaagagctgcaaaaagcgcctacccttcggtcgctgcgctccctacgccccgccgcttcgcgtcggcctatcgcggccgctggccgctcaaaaatggctggcctacggccaggcaatctaccagggcgcggacaagccgcgccgtcgccactcgaccgccggcgcccacatcaaggcaccggtgggtatgcctgacgatgcgtggagaccgaaaccttgcgctcgttcgccagccaggacagaaatgcctcgacttcgctgctgcccaaggttgccgggtgacgcacaccgtggaaacggatgaaggcacgaacccagtggacataagcctgttcggttcgtaagctgtaatgcaagtagcgtatgcgctcacgcaactggtccagaaccttgaccgaacgcagcggtggtaacggcgcagtggcggttttcatggcttgttatgactgtttttttggggtacagtctatgcctcgggcatccaagcagcaagcgcgttacgccgtgggtcgatgtttgatgttatggagcagcaacgatgttacgcagcagggcagtcgccctaaaacaaagttaaacatcatgagggaagcggtgatcgccgaagtatcgactcaactatcagaggtagttggcgtcatcgagcgccatctcgaaccgacgttgctggccgtacatttgtacggctccgcagtggatggcggcctgaagccacacagtgatattgatttgctggttacggtgaccgtaaggcttgatgaaacaacgcggcgagctttgatcaacgaccttttggaaacttcggcttcccctggagagagcgagattctccgcgctgtagaagtcaccattgttgtgcacgacgacatcattccgtggcgttatccagctaagcgcgaactgcaatttggagaatggcagcgcaatgacattcttgcaggtatcttcgagccagccacgatcgacattgatctggctatcttgctgacaaaagcaagagaacatagcgttgccttggtaggtccagcggcggaggaactctttgatccggttcctgaacaggatctatttgaggcgctaaatgaaaccttaacgctatggaactcgccgcccgactgggctggcgatgagcgaaatgtagtgcttacgttgtcccgcatttggtacagcgcagtaaccggcaaaatcgcgccgaaggatgtcgctgccgactgggcaatggagcgcctgccggcccagtatcagcccgtcatacttgaagctagacaggcttatcttggacaagaagaagatcgcttggcctcgcgcgcagatcagttggaagaatttgtccactacgtgaaaggcgagatcaccaaggtagtcggcaaataatgtctaacaattcgttcaagccgacgccgcttcgcggcgcggcttaactcaagcgttagatgcactaagcacataattgctcacagccaaactatcaggtcaagtctgcttttattatttttaagcgtgcataataagccctacacaaattgggagatatatcatgaaaggctggctttttcttgttatcgcaatagttggcgaagtaatcgcaacatagcttgcttggtcgttccgcgtgaacgtcggctcgattgtacctgcgttcaaatactttgcgatcgtgttgcgcgcctgcccggtgcgtcggctgatctcacggatcgactgcttctctcgcaacgccatccgacggatgatgtttaaaagtcccatgtggatcactccgttgccccgtcgctcaccgtgttggggggaaggtgcacatggctcagttctcaatggaaattatctgcctaaccggctcagttctgcgtagaaaccaacatgcaagctccaccgggtgcaaagcggcagcggcggcaggatatattcaattgtaaatggcttcatgtccgggaaatctacatggatcagcaatgagtatgatggtcaatatggagaaaaagaaagagtaattaccaattttttttcaattcaaaaatgtagatgtccgcagcgttattataaaatgaaagtacattttgataaaacgacaaattacgatccgtcgtatttataggcgaaagcaataaacaaattattctaattcggaaatctttatttcgacgtgtctacattcacgtccaaatgggggcttagatgagaaacttcacgatcggctctagttcgagcgatctagtaacatagatgacaccgcgcgcgataatttatcctagtttgcgcgctatattttgttttctatcgcgtattaaatgtataattgcgggactctaatcataaaaacccatctcataaataacgtcatgcattacatgttaattattacatgcttaacgtaattcaacagaaattatatgataatcatcgcaagaccggcaacaggattcaatcttaagaaactttattgccaaatgtttgaacgatcggggaaattcgtttctatgcttcaattctgctctatagatgttcttctagtcttaacttttagaaggcacaacatttgaaatgttggtaatttttctgctgggtagtgaaccattgtaatttgtgtttgcttatattatccgttgggtttctctatgttatctgtggggccatatcccagaactggttgagtcggtccaacacctgggtgccaatcatgtcgatggtggggtatggtccggattgaaagaaatatagtttaaatatttattgataaaataacaagtcaggtattatagtccaagcaaaaacataaatttattgatgcaagtttaaattcagaaatatttcaataactgattatatcagctggtacattgccgtagatgaaagactgagtgcgatattatgtgtaatacataaattgatgatatagctagcttagctcatcgggtcagaagaactcgtcaagaaggcgatagaaggcgatgcgctgcgaatcgggagcggcgataccgtaaagcacgaggaagcggtcagcccattcgccgccaagctcttcagcaatatcacgggtagccaacgctatgtcctgatagcggtccgccacacccagccggccacagtcgatgaatccagaaaagcggccattttccaccatgatattcggcaagcaggcatcgccatgagtcacgacgagatcctcgccgtcgggcatgcgcgccttgagcctggcgaacagttcggctggcgcgagcccctgatgctcttcgtccagatcatcctgatcgacaagaccggcttccatccgagtacgtgctcgctcgatgcgatgtttcgcttggtggtcgaatgggcaggtagccggatcaagcgtatgcagccgccgcattgcatcagccatgatggatactttctcggcaggagcaaggtgagatgacaggagatcctgccccggcacttcgcccaatagcagccagtcccttcccgcttcagtgacaacgtcgagcacagctgcgcaaggaacgcccgtcgtggccagccacgatagccgcgctgcctcgtcctgaagttcattcagggcaccggacaggtcggtcttgacaaaaagaaccgggcgcccctgcgctgacagccggaacacggcggcatcagagcagccgattgtctgttgtgcccagtcatagccgaatagcctctccacccaagcggccggagaacctgcgtgcaatccatcttgttcaatccaagctcccattttctgtgattttggatgtgtttttgtatggattgagagtgaatatgagactctaattggataccgaggggaatttatggaacgtcagtggagcatttttgacaagaaatatttgctagctgatagtgaccttaggcgacttttgaacgcgcaataatggtttctgacgtatgtgcttagctcattaaactccagaaacccgcggctgagtggctccttcaacgttgcggttctgtcagttccaaacgtaaaacggcttgtcccgcgtcatcggcgggggtcattccggactgtggggccatatcccagaactggttgagtcggtccaacacctgggtgccaatcatgtcgatggtggggtatggccaattttttttcaattcaaaaatgtagatgtccgcagcgttattataaaatgaaagtacattttgataaaacgacaaattacgatccgtcgtatttataggcgaaagcaataaacaaattattctaattcggaaatctttatttcgacgtgtctacattcacgtccaaatgggggcttagatgagaaacttcacgatcggctctagaggccatgg

SEQ ID NO: 6 - DNA, 801 bp, Artificial Sequence
  Neomycin phosphotransferase
atgggagcttggattgaacaagatggattgcacgcaggttctccggccgcttgggtggagaggctattcggctatgactgggcacaacagacaatcggctgctctgatgccgccgtgttccggctgtcagcgcaggggcgcccggttctttttgtcaagaccgacctgtccggtgccctgaatgaacttcaggacgaggcagcgcggctatcgtggctggccacgacgggcgttccttgcgcagctgtgctcgacgttgtcactgaagcgggaagggactggctgctattgggcgaagtgccggggcaggatctcctgtcatctcaccttgctcctgccgagaaagtatccatcatggctgatgcaatgcggcggctgcatacgcttgatccggctacctgcccattcgaccaccaagcgaaacatcgcatcgagcgagcacgtactcggatggaagccggtcttgtcgatcaggatgatctggacgaagagcatcaggggctcgcgccagccgaactgttcgccaggctcaaggcgcgcatgcccgacggcgaggatctcgtcgtgactcatggcgatgcctgcttgccgaatatcatggtggaaaatggccgcttttctggattcatcgactgtggccggctgggtgtggcggaccgctatcaggacatagcgttggctacccgtgatattgctgaagagcttggcggcgaatgggctgaccgcttcctcgtgctttacggtatcgccgctcccgattcgcagcgcatcgccttctatcgccttcttgacgagttcttc

SEQ ID NO: 7 - DNA, 702 bp, Artificial Sequence
  tdTomato, orange fluorescent protein
atggtgagcaagggcgaggaggtcatcaaagagttcatgcgcttcaaggtgcgcatggagggctccatgaacggccacgagttcgagatcgagggcgagggcgagggccgcccctacgagggcacccagaccgccaagctgaaggtgaccaagggcggccccctgcccttcgcctgggacatcctgtccccccagttcatgtacggctccaaggcgtacgtgaagcaccccgccgacatccccgattacaagaagctgtccttccccgagggcttcaagtgggagcgcgtgatgaacttcgaggacggcggtctggtgaccgtgacccaggactcctccctgcaggacggcacgctgatctacaaggtgaagatgcgcggcaccaacttcccccccgacggccccgtaatgcagaagaagaccatgggctgggaggcctccaccgagcgcctgtacccccgcgacggcgtgctgaagggcgagatccaccaggccctgaagctgaaggacggcggccactacctggtggagttcaagaccatctacatggccaagaagcccgtgcaactgcccggctactactacgtggacaccaagctggacatcacctcccacaacgaggactacaccatcgtggaacagtacgagcgctccgagggccgccaccacctgttcctgtacggcatggacgagctgtacaag

SEQ ID NO: 8 - DNA, 691 bp, Artificial Sequence
  double 35s promoter
gttcagaagaccagagggctattgagacttttcaacaaagggtaatatcgggaaacctcctcggattccattgcccagctatctgtcacttcatcgaaaggacagtagaaaaggaagatggcttctacaaatgccatcattgcgataaaggaaaggctatcgttcaagatgcctctaccgacagtggtcccaaagatggacccccacccacgaggaacatcgtggaaaaagaagacgttccaaccacgtcttcaaagcaagtggattgatgtgatacatggtggagcacgacactctcgtctactccaagaatatcaaagatacagtctcagaagaccagagggctattgagacttttcaacaaagggtaatatcgggaaacctcctcggattccattgcccagctatctgtcacttcatcgaaaggacagtagaaaaggaagatggcttctacaaatgccatcattgcgataaaggaaaggctatcgttcaagatgcctctaccgacagtggtcccaaagatggacccccacccacgaggaacatcgtggaaaaagaagacgttccaaccacgtcttcaaagcaagtggattgatgtgatatctccactgacgtaagggatgacgcacaatcccactatccttcgcaagacccttcctctatataaggaagttcatttcatttggagagg

SEQ ID NO: 9 - DNA, 698 bp, Artificial Sequence
  Col E1 origin of replication
aaaaggatctaggtgaagatcctttttgataatctcatgaccaaaatcccttaacgtgagttttcgttccactgagcgtcagaccccgtagaaaagatcaaaggatcttcttgagatcctttttttctgcgcgtaatctgctgcttgcaaacaaaaaaaccaccgctaccagcggtggtttgtttgccggatcaagagctaccaactctttttccgaaggtaactggcttcagcagagcgcagataccaaatactgttcttctagtgtagccgtagttaggccaccacttcaagaactctgtagcaccgcctacatacctcgctctgctaatcctgttaccagtggctgctgccagtggcgataagtcgtgtcttaccgggttggactcaagacgatagttaccggataaggcgcagcggtcgggctgaacggggggttcgtgcacacagcccagcttggagcgaacgacctacaccgaactgagatacctacagcgtgagctatgagaaagcgccacgcttcccgaagggagaaaggcggacaggtatccggtaagcggcagggtcggaacaggagagcgcacgagggagcttccagggggaaacgcctggtatctttatagtcctgtcgggtttcgccacctctgacttgagcgtcgatttttgtgatgctcgtcaggggggcggagcctatggaa

SEQ ID NO: 10 - DNA, 3706 bp, Artificial Sequence
  pVS1 Replicon
cgacatgtcgcacaagtcctaagttacgcgacaggctgccgccctgcccttttcctggcgttttcttgtcgcgtgttttagtcgcataaagtagaatacttgcgactagaaccggagacattacgccatgaacaagagcgccgccgctggcctgctgggctatgcccgcgtcagcaccgacgaccaggacttgaccaaccaacgggccgaactgcacgcggccggctgcaccaagctgttttccgagaagatcaccggcaccaggcgcgaccgcccggagctggccaggatgcttgaccacctacgccctggcgacgttgtgacagtgaccaggctagaccgcctggcccgcagcacccgcgacctactggacattgccgagcgcatccaggaggccggcgcgggcctgcgtagcctggcagagccgtgggccgacaccaccacgccggccggccgcatggtgttgaccgtgttcgccggcattgccgagttcgagcgttccctaatcatcgaccgcacccggagcgggcgcgaggccgccaaggcgcgaggcgtgaagtttggcccccgccctaccctcaccccggcacagatcgcgcacgcccgcgagctgatcgaccaggaaggccgcaccgtgaaagaggcggctgcactgcttggcgtgcatcgctcgaccctgtaccgcgcacttgagcgcagcgaggaagtgacgcccaccgaggccaggcggcgcggtgccttccgtgaggacgcattgaccgaggccgacgccctggcggccgccgagaatgaacgccaagaggaacaagcatgaaaccgcaccaggacggccaggacgaaccgtttttcattaccgaagagatcgaggcggagatgatcgcggccgggtacgtgttcgagccgcccgcgcacgtctcaaccgtgcggctgcatgaaatcctggccggtttgtctgatgccaagctcgcggcctggccggcgagcttggccgctgaagaaaccgagcgccgccgtctaaaaaggtgatgtgtatttgagtaaaacagcttgcgtcatgcggtcgctgcgtatatgatgcgatgagtaaataaacaaatacgcaaggggaacgcatgaaggttatcgctgtacttaaccagaaaggcgggtcaggcaagacgaccatcgcaacccatctagcccgcgccctgcaactcgccggggccgatgttctgttagtcgattccgatccccagggcagtgcccgcgattgggcggccgtgcgggaagatcaaccgctaaccgttgtcggcatcgaccgcccgacgattgaccgcgacgtgaaggccatcggccggcgcgacttcgtagtgatcgacggagcgccccaggcggcggacttggctgtgtccgcgatcaaggcagccgacttcgtgctgattccggtgcagccaagcccttacgacatatgggccaccgccgacctggtggagctggttaagcagcgcattgaggtcacggatggaaggctacaagcggcctttgtcgtgtcgcgggcgatcaaaggcacgcgcatcggcggtgaggttgccgaggcgctggccgggtacgagctgcccattcttgagtcccgtatcacgcagcgcgtgagctacccaggcactgccgccgccggcacaaccgttcttgaatcagaacccgagggcgacgctgcccgcgaggtccaggcgctggccgctgaaattaaatcaaaactcatttgagttaatgaggtaaagagaaaatgagcaaaagcacaaacacgctaagtgccggccgtccgagcgcacgcagcagcaaggctgcaacgttggccagcctggcagacacgccagccatgaagcgggtcaactttcagttgccggcggaggatcacaccaagctgaagatgtacgcggtacgccaaggcaagaccattaccgagctgctatctgaatacatcgcgcagctaccagagtaaatgagcaaatgaataaatgagtagatgaattttagcggctaaaggaggcggcatggaaaatcaagaacaaccaggcaccgacgccgtggaatgccccatgtgtggaggaacgggcggttggccaggcgtaagcggctgggttgtctgccggccctgcaatggcactggaacccccaagcccgaggaatcggcgtgagcggtcgcaaaccatccggcccggtacaaatcggcgcggcgctgggtgatgacctggtggagaagttgaaggcggcgcaggccgcccagcggcaacgcatcgaggcagaagcacgccccggtgaatcgtggcaagcggccgctgatcgaatccgcaaagaatcccggcaaccgccggcagccggtgcgccgtcgattaggaagccgcccaagggcgacgagcaaccagattttttcgttccgatgctctatgacgtgggcacccgcgatagtcgcagcatcatggacgtggccgttttccgtctgtcgaagcgtgaccgacgagctggcgaggtgatccgctacgagcttccagacgggcacgtagaggtttccgcagggccggccggcatggcgagtgtgtgggattacgacctggtactgatggcggtttcccatctaaccgaatccatgaaccgataccgggaagggaagggagacaagcccggccgcgtgttccgtccacacgttgcggacgtactcaagttctgccggcgagccgatggcggaaagcagaaagacgacctggtagaaacctgcattcggttaaacaccacgcacgttgccatgcagcgtacgaagaaggccaagaacggccgcctggtgacggtatccgagggtgaagccttgattagccgctacaagatcgtaaagagcgaaaccgggcggccggagtacatcgagatcgagctagctgattggatgtaccgcgagatcacagaaggcaagaacccggacgtgctgacggttcaccccgattactttttgatcgatcccggcatcggccgttttctctaccgcctggcacgccgcgccgcaggcaaggcagaagccagatggttgttcaagacgatctacgaacgcagtggcagcgccggagagttcaagaagttctgtttcaccgtgcgcaagctgatcgggtcaaatgacctgccggagtacgatttgaaggaggaggcggggcaggctggcccgatcctagtcatgcgctaccgcaacctgatcgagggcgaagcatccgccggttcctaatgtacggagcagatgctagggcaaattgccctagcaggggaaaaaggtcgaaaaggtctctttcctgtggatagcacgtacattgggaacccaaagccgtacattgggaaccggaacccgtacattgggaacccaaagccgtacattgggaaccggtcacacatgtaagtgactgatataaaagagaaaaaaggcgatttttccgcctaaaactctttaaaacttattaaaactcttaaaacccgcctggcctgtgcataactgtctggccagcgcacagccgaagagctgcaaaaagcgcctacccttcggtcgctgcgctccctacgccccgccgcttcgcgtcggcctatcgcggccgctggccgctcaaaaatggctggcctacggccaggcaatctaccagggcgcggacaagccgcgccgtcgccactcgaccgccggcgcccacatcaaggcacc

SEQ ID NO: 11 - DNA, 1008 bp, Escherichia coli
atgcgctcacgcaactggtccagaaccttgaccgaacgcagcggtggtaacggcgcagtggcggttttcatggcttgttatgactgtttttttggggtacagtctatgcctcgggcatccaagcagcaagcgcgttacgccgtgggtcgatgtttgatgttatggagcagcaacgatgttacgcagcagggcagtcgccctaaaacaaagttaaacatcatgagggaagcggtgatcgccgaagtatcgactcaactatcagaggtagttggcgtcatcgagcgccatctcgaaccgacgttgctggccgtacatttgtacggctccgcagtggatggcggcctgaagccacacagtgatattgatttgctggttacggtgaccgtaaggcttgatgaaacaacgcggcgagctttgatcaacgaccttttggaaacttcggcttcccctggagagagcgagattctccgcgctgtagaagtcaccattgttgtgcacgacgacatcattccgtggcgttatccagctaagcgcgaactgcaatttggagaatggcagcgcaatgacattcttgcaggtatcttcgagccagccacgatcgacattgatctggctatcttgctgacaaaagcaagagaacatagcgttgccttggtaggtccagcggcggaggaactctttgatccggttcctgaacaggatctatttgaggcgctaaatgaaaccttaacgctatggaactcgccgcccgactgggctggcgatgagcgaaatgtagtgcttacgttgtcccgcatttggtacagcgcagtaaccggcaaaatcgcgccgaaggatgtcgctgccgactgggcaatggagcgcctgccggcccagtatcagcccgtcatacttgaagctagacaggcttatcttggacaagaagaagatcgcttggcctcgcgcgcagatcagttggaagaatttgtccactacgtgaaaggcgagatcaccaaggtagtcggcaaa

SEQ ID NO: 12 - DNA, 909 bp, Artificial Sequence
  cDNA sequence of ZmWUS2
atggcggccaatgcgggcggcggtggagcgggaggaggcagcggcagcggcagcgtggctgcgccggcggtgtgccgccccagcggctcgcggtggacgccgacgccggagcagatcaggatgctgaaggagctctactacggctgcggcatccggtcgcccagctcggagcagatccagcgcatcaccgccatgctgcggcagcacggcaagatcgagggcaagaacgtcttctactggttccagaaccacaaggcccgcgagcgccagaagcgccgcctcaccagcctcgacgtcaacgtgcccgccgccggcgcggccgacgccaccaccagccaactcggcgtcctctcgctgtcgtcgccgccgccttcaggcgcggcgcctccctcgcccaccctcggcttctacgccgccggcaatggcggcggatcggctgtgctgctggacacgagttccgactggggcagcagcggcgctgccatggccaccgagacatgcttcctccaggactacatgggcgtgacggacacgggcagctcgtcgcagtggccacgcttctcgtcgtcggacacgataatggcggcggccgcggcgcgggcggcgacgacgcgggcgcccgagacgctccctctcttcccgacctgcggcgacgacggcggcagcggtagcagcagctacttgccgttctggggtgccgcgtccacaactgccggcgccacttcttccgttgcgatccagcagcaacaccagctgcaggagcagtacagcttttacagcaacagcaacagcacccagctggccggcaccggcaaccaagacgtatcggcaacagcagcagcagccgccgccctggagctgagcctcagctcatggtgctccccttaccctgctgcagggagtatgtga

SEQ ID NO: 13 - protein, 302 aa, Zea mays
MAANAGGGGAGGGSGSGSVAAPAVCRPSGSRWTPTPEQIRMLKELYYGCGIRSPSSEQIQRITAMLRQHGKIEGKNVFYWFQNHKARERQKRRLTSLDVNVPAAGAADATTSQLGVLSLSSPPPSGAAPPSPTLGFYAAGNGGGSAVLLDTSSDWGSSGAAMATETCFLQDYMGVTDTGSSSQWPRFSSSDTIMAAAAARAATTRAPETLPLFPTCGDDGGSGSSSYLPFWGAASTTAGATSSVAIQQQHQLQEQYSFYSNSNSTQLAGTGNQDVSATAAAAAALELSLSSWCSPYPAAGSM

SEQ ID NO: 14 - DNA, 13362 bp, Artificial Sequence
  IPR232-pS-01
ccggattgaaagaaatatagtttaaatatttattgataaaataacaagtcaggtattatagtccaagcaaaaacataaatttattgatgcaagtttaaattcagaaatatttcaataactgattatatcagctggtacattgccgtagatgaaagactgagtgcgatattatgtgtaatacataaattgatgatatagctagcttagctcatcgggtcagaagaactcgtcaagaaggcgatagaaggcgatgcgctgcgaatcgggagcggcgataccgtaaagcacgaggaagcggtcagcccattcgccgccaagctcttcagcaatatcacgggtagccaacgctatgtcctgatagcggtccgccacacccagccggccacagtcgatgaatccagaaaagcggccattttccaccatgatattcggcaagcaggcatcgccatgagtcacgacgagatcctcgccgtcgggcatgcgcgccttgagcctggcgaacagttcggctggcgcgagcccctgatgctcttcgtccagatcatcctgatcgacaagaccggcttccatccgagtacgtgctcgctcgatgcgatgtttcgcttggtggtcgaatgggcaggtagccggatcaagcgtatgcagccgccgcattgcatcagccatgatggatactttctcggcaggagcaaggtgagatgacaggagatcctgccccggcacttcgcccaatagcagccagtcccttcccgcttcagtgacaacgtcgagcacagctgcgcaaggaacgcccgtcgtggccagccacgatagccgcgctgcctcgtcctgaagttcattcagggcaccggacaggtcggtcttgacaaaaagaaccgggcgcccctgcgctgacagccggaacacggcggcatcagagcagccgattgtctgttgtgcccagtcatagccgaatagcctctccacccaagcggccggagaacctgcgtgcaatccatcttgttcaatccaagctcccattttctgtgattttggatgtgtttttgtatggattgagagtgaatatgagactctaattggataccgaggggaatttatggaacgtcagtggagcatttttgacaagaaatatttgctagctgatagtgaccttaggcgacttttgaacgcgcaataatggtttctgacgtatgtgcttagctcattaaactccagaaacccgcggctgagtggctccttcaacgttgcggttctgtcagttccaaacgtaaaacggcttgtcccgcgtcatcggcgggggtcattccggactgtggggccatatcccagaactggttgagtcggtccaacacctgggtgccaatcatgtcgatggtggggtatggccaattttttttcaattcaaaaatgtagatgtccgcagcgttattataaaatgaaagtacattttgataaaacgacaaattacgatccgtcgtatttataggcgaaagcaataaacaaattattctaattcggaaatctttatttcgacgtgtctacattcacgtccaaatgggggcttagatgagaaacttcacgatcggctctagaggccatggcggccggaagacaaagatagcccggggcctgcaggaccaatgcattggatctggagacccgccggcggcagaagagatccaacaaaacattcacaatggattatagaaacatttgtttattcattataatgagatcttacattcatttaatattagaaaaagccacaaattcataacacaacaagccaagaaaaaaacacaaacttaagcacacaagctttttatttgacacaccaaatatttcatcttcatcttcatatgagctcgtcgacggtaccccctcaattagttacatcaccactttgtacaagaaagctgggtgtcatttttgatgaaacaggagctttttgatatttccatttgaatattttggtatctgattagtgatgatttcagctaacatctctgggaactcaatactcatggtcttatccaaaaatgtctggaagcagtaggtaaggagattctcaaccacctcatgcatggagtccagaagctttgtcagttggtaaaaccgttgccagttctgactggagttcccttcccttttgacgatggcttttcctagctctttgatataagtcattcgaatctcatcaaataactcttggctcttcagaccttccttaggaactgaggagagaagcagtaaggttttcatacagagatactcttcataggatacctgcaatctttgtaattcagaggagacaaacagcatgtgtttacattggtcatacatgcagggtagagacattctctgctcattaataatcagatcaggagcaaagcagagcaggtttccacttgattgtctgtatgatctccaacccagggcaaatgccatgagaaacatccatgagtactgtagcagggtcatttggtcatccaggtgtaagtttctgaagcctggtatcgcctttgcccatttcactgctgcaatcacttgacgcccacctaacatgttgagtgtggtcataattctccacgctgaatctggaacagagctatcatatcctgcatacaacacctcgggttcaatcacctccagcagtgacaccaaggtaggggtgagctgtggtaatgcagcaggaactattgttttgttaggattttccgaagtgtcttgtgagactcctgcagtggcttgctgaatccctttgatttttttctttgtagatccattgtcgttccaaactgtaaatgttggagcaacttctccaccaccttccccatggtaatacatattagagccaacattattcgtcattgccgcgggaaaatctccacctggcgactgctgggtctgctgctgctgagcaaagtaataatggtttcttgcgttataatcaaactcactagcagcgtaggcatcgcagttaaccggggctgcaaatccttgataaccaccataaccaacaacatttccacaaacagtaaccgaatcatccgaaacagaactttgatgatcgatattagtcatgaggctctgcgtgttgctcaagaaatggtgttgatcatcctcttgtttgaaacaagccctagcactctccgaagacaagtttcctccattgtaataataaccattgtacctctcttgatgttggtgcaataagctcaaatctactccctgatgatgctgaaccgcagcgttttgccaaccgctagcactattctcactctctgaaacgttattactgatcatcatcatacttggaaccggacggttagcctccttgagacgttttgcggcgctaccaataggaagactagggctttcgaggattgctttaacgttgtatctgttcatgtcgaagttagtcactgcggttaatcctctgaatttgatggccgcaatgtcgtatgcctctgcagcttcttcttgtgtgccaaaagttcccaagtagaggtctttgttaccggcgactcttcctatcctagcttgccatcttccatgttggtgatgtcttgttactccacgataaatcgatgcaccacgagagaaaccactacttttcctgcgcagtgaggcaacatactcttgccttgtcatgtgcttcatctcttctacctctttttcatattcgctcatggggaagttagtagtagtggtggttccccaatacttgagtgcggctaaatcataagccctagctgctttttcttctttgtcataacctcccaaataaacttgtcttcctttgcgcgtttggccttctcttttacaactattatcccataaatgtgcctcatatcttcctgtccaccgatgccttgtaacaccgcggtatatagacgtcctctgtccaaaactctcaatagttttcttcggtgtagcttcaacgctatcatcaatagtcttcccttgggcaacaacgttgttattgctgtcgttgttgttatcacaagaagtagatgagttcattgagagggacaggccttttgcagcattgccattttcttgattatcaacattatccacgggttgatttctcagccatgtctttatcatcgaaagtcctagtgagccaccaccaccgtctcctcctccataacagccacttccacttccatctccaacgttttcgttggtgttgtaaatcgtggtggtgcggccaaggaaattctcaagctttggtccatcttgctcatcgttgtggatgttattgcatgcacaaccattgatgtcccaatctcgggagtgactattgttgtctctggtgaaagcatcgacgacgacaccaaagggagaaggaaacgatgtttggatggctgaagactcatcggaggcagcggtcggatcgtaacagtactctccggcgacatctacgacggttgtggtggtggaagagtagacgtccttacgatggtgattttgttcataaggagagagagaaaagcctaaccagttattatccattgagcctgcttttttgtacaaacttgtgatcgggatctgtaattgtaatgttgtttgttgtttgttgttgttggtaattgtggatcctctagagtcccccgtgttctctccaaatgaaatgaacttccttatatagaggaagggtcttgcgaaggatagtgggattgtgcgtcatcccttacgtcagtggagatatcacatcaatccacttgctttgaagacgtggttggaacgtcttctttttccacgatgctcctcgtgggtgggggtccatctttgggaccactgtcggcagaggcatcttcaacgatggcctttcctttatcgcaatgatggcatttgtaggagccaccttccttttccactatcttcacaataaagtgacagatagctgggcaatggaatccgaggaggtttccggatattaccctttgttgaaaagtctcaattgccctttggtcttctgagactgtatctttgatatttttggagtagacaagtgtgtcgtgctccaccatgttgacgaagattttcttcttgtcattgagtcgtaagagactctgtatgaactgttcgccagtctttacggcgagttctgttaggtcctctatttgaatctttgactccatggcctttgattcagtgggaactacctttttagagactccaatctctattacttgcctcgccggcgggtctcgggatcccctgcaggactagtggatttgtcttcaaggccttaagggccagatcttgggcccggtacccgatcagattgtcgtttcccgccttcggtttaaactatcagtgtttgacaggatatattggcgggtaaacctaagagaaaagagcgtttattagaataatcggatatttaaaagggcgtgaaaaggtttatccgttcgtccatttgtatgtgcatgccaaccacagggttcccctcgggagtgcttggcattccgtgcgataatgacttctgttcaaccacccaaacgtcggaaagcctgacgacggagcagcattccaaaaagatcccttggctcgtctgggtcggctagaaggtcgagtgggctgctgtggcttgatccctcaacgcggtcgcggacgtagcgcagcgccgaaaaatcctcgatcgcaaatccgacgctgtcgaaaagcgtgatctgcttgtcgctctttcggccgacgtcctggccagtcatcacgcgccaaagttccgtcacaggatgatctggcgcgagttgctggatctcgccttcaatccgggtctgtggcgggaactccacgaaaatatccgaacgcagcaagatatcgcggtgcatctcggtcttgcctgggcagtcgccgccgacgccgttgatgtggacgccgaaaaggatctaggtgaagatcctttttgataatctcatgaccaaaatcccttaacgtgagttttcgttccactgagcgtcagaccccgtagaaaagatcaaaggatcttcttgagatcctttttttctgcgcgtaatctgctgcttgcaaacaaaaaaaccaccgctaccagcggtggtttgtttgccggatcaagagctaccaactctttttccgaaggtaactggcttcagcagagcgcagataccaaatactgttcttctagtgtagccgtagttaggccaccacttcaagaactctgtagcaccgcctacatacctcgctctgctaatcctgttaccagtggctgctgccagtggcgataagtcgtgtcttaccgggttggactcaagacgatagttaccggataaggcgcagcggtcgggctgaacggggggttcgtgcacacagcccagcttggagcgaacgacctacaccgaactgagatacctacagcgtgagctatgagaaagcgccacgcttcccgaagggagaaaggcggacaggtatccggtaagcggcagggtcggaacaggagagcgcacgagggagcttccagggggaaacgcctggtatctttatagtcctgtcgggtttcgccacctctgacttgagcgtcgatttttgtgatgctcgtcaggggggcggagcctatggaaaaacgccagcaacgcggcctttttacggttcctggccttttgctggccttttgctcacatgttctttcctgcgttatcccctgattctgtggataaccgattaccgcctttgagtgagctgataccgctcgccgcagccgaacgaccgagcgcagcgagtcagtgagcgaggaagcggaagagcgcctgatgcggtattttctccttacgcatctgtgcggtatttcacaccgcatatggtgcactctcagtacaatctgctctgatgccgcatagttaagccagtatacactccgctatcgctacgtgactgggtcatggctgcgccccgacacccgccaacacccgctgacgcgccctgacgggcttgtctgctcccggcatccgcttacagacaagctgtgaccgtctccgggagctgcatgtgtcagaggttttcaccgtcatcaccgaaacgcgcgaggcaggggtacgtcgaggtcgatccaacccctccgctgctatagtgcagtcggcttctgacgttcagtgcagccgtcttctgaaaacgacatgtcgcacaagtcctaagttacgcgacaggctgccgccctgcccttttcctggcgttttcttgtcgcgtgttttagtcgcataaagtagaatacttgcgactagaaccggagacattacgccatgaacaagagcgccgccgctggcctgctgggctatgcccgcgtcagcaccgacgaccaggacttgaccaaccaacgggccgaactgcacgcggccggctgcaccaagctgttttccgagaagatcaccggcaccaggcgcgaccgcccggagctggccaggatgcttgaccacctacgccctggcgacgttgtgacagtgaccaggctagaccgcctggcccgcagcacccgcgacctactggacattgccgagcacatccaggaggccggcgcgggcctgcgtagcctggcagagccgtgggccgacaccaccacgccggccggccgcatggtgttgaccgtgttcgccggcattgccgagttcgagcgttccctaatcatcgaccgcacccggagcgggcgcgaggccgccaaggcgcgaggcgtgaagtttggcccccgccctaccctcaccccggcacagatcgcgcacgcccgcgagctgatcgaccaggaaggccgcaccgtgaaagaggcggctgcactgcttggcgtgcatcgctcgaccctgtaccgcgcacttgagcgcagcgaggaagtgacgcccaccgaggccaggcggcgcggtgccttccgtgaggacgcattgaccgaggccgacgccctggcggccgccgagaatgaacgccaagaggaacaagcatgaaaccgcaccaggacggccaggacgaaccgtttttcattaccgaagagatcgaggcggagatgatcgcggccgggtacgtgttcgagccgcccgcgcacgtctcaaccgtgcggctgcatgaaatcctggccggtttgtctgatgccaagctcgcggcctggccggcgagcttggccgctgaagaaaccgagcgccgccgtctaaaaaggtgatgtgtatttgagtaaaacagcttgcgtcatgcggtcgctgcgtatatgatgcgatgagtaaataaacaaatacgcaaggggaacgcatgaaggttatcgctgtacttaaccagaaaggcgggtcaggcaagacgaccatcgcaacccatctagcccgcgccctgcaactcgccggggccgatgttctgttagtcgattccgatccccagggcagtgcccgcgattgggcggccgtgcgggaagatcaaccgctaaccgttgtcggcatcgaccgcccgacgattgaccgcgacgtgaaggccatcggccggcgcgacttcgtagtgatcgacggagcgccccaggcggcggacttggctgtgtccgcgatcaaggcagccgacttcgtgctgattccggtgcagccaagcccttacgacatatgggccaccgccgacctggtggagctggttaagcagcgcattgaggtcacggatggaaggctacaagcggcctttgtcgtgtcgcgggcgatcaaaggcacgcgcatcggcggtgaggttgccgaggcgctggccgggtacgagctgcccattcttgagtcccgtatcacgcagcgcgtgagctacccaggcactgccgccgccggcacaaccgttcttgaatcagaacccgagggcgacgctgcccgcgaggtccaggcgctggccgctgaaattaaatcaaaactcatttgagttaatgaggtaaagagaaaatgagcaaaagcacaaacacgctaagtgccggccgtccgagcgcacgcagcagcaaggctgcaacgttggccagcctggcagacacgccagccatgaagcgggtcaactttcagttgccggcggaggatcacaccaagctgaagatgtacgcggtacgccaaggcaagaccattaccgagctgctatctgaatacatcgcgcagctaccagagtaaatgagcaaatgaataaatgagtagatgaattttagcggctaaaggaggcggcatggaaaatcaagaacaaccaggcaccgacgccgtggaatgccccatgtgtggaggaacgggcggttggccaggcgtaagcggctgggttgtctgccggccctgcaatggcactggaacccccaagcccgaggaatcggcgtgagcggtcgcaaaccatccggcccggtacaaatcggcgcggcgctgggtgatgacctggtggagaagttgaaggcggcgcaggccgcccagcggcaacgcatcgaggcagaagcacgccccggtgaatcgtggcaagcggccgctgatcgaatccgcaaagaatcccggcaaccgccggcagccggtgcgccgtcgattaggaagccgcccaagggcgacgagcaaccagattttttcgttccgatgctctatgacgtgggcacccgcgatagtcgcagcatcatggacgtggccgttttccgtctgtcgaagcgtgaccgacgagctggcgaggtgatccgctacgagcttccagacgggcacgtagaggtttccgcagggccggccggcatggcgagtgtgtgggattacgacctggtactgatggcggtttcccatctaaccgaatccatgaaccgataccgggaagggaagggagacaagcccggccgcgtgttccgtccacacgttgcggacgtactcaagttctgccggcgagccgatggcggaaagcagaaagacgacctggtagaaacctgcattcggttaaacaccacgcacgttgccatgcagcgtacgaagaaggccaagaacggccgcctggtgacggtatccgagggtgaagccttgattagccgctacaagatcgtaaagagcgaaaccgggcggccggagtacatcgagatcgagctagctgattggatgtaccgcgagatcacagaaggcaagaacccggacgtgctgacggttcaccccgattactttttgatcgatcccggcatcggccgttttctctaccgcctggcacgccgcgccgcaggcaaggcagaagccagatggttgttcaagacgatctacgaacgcagtggcagcgccggagagttcaagaagttctgtttcaccgtgcgcaagctgatcgggtcaaatgacctgccggagtacgatttgaaggaggaggcggggcaggctggcccgatcctagtcatgcgctaccgcaacctgatcgaaggcgaagcatccgccggttcctaatgtacggagcagatgctagggcaaattgccctagcaggggaaaaaggtcgaaaaggtctctttcctgtggatagcacgtacattgggaacccaaagccgtacattgggaaccggaacccgtacattgggaacccaaagccgtacattgggaaccggtcacacatgtaagtgactgatataaaagagaaaaaaggcgatttttccgcctaaaactctttaaaacttattaaaactcttaaaacccgcctggcctgtgcataactgtctggccagcgcacagccgaagagctgcaaaaagcgcctacccttcggtcgctgcgctccctacgccccgccgcttcgcgtcggcctatcgcggccgctggccgctcaaaaatggctggcctacggccaggcaatctaccagggcgcggacaagccgcgccgtcgccactcgaccgccggcgcccacatcaaggcaccggtgggtatgcctgacgatgcgtggagaccgaaaccttgcgctcgttcgccagccaggacagaaatgcctcgacttcgctgctgcccaaggttgccgggtgacgcacaccgtggaaacggatgaaggcacgaacccagtggacataagcctgttcggttcgtaagctgtaatgcaagtagcgtatgcgctcacgcaactggtccagaaccttgaccgaacgcagcggtggtaacggcgcagtggcggttttcatggcttgttatgactgtttttttggggtacagtctatgcctcgggcatccaagcagcaagcgcgttacgccgtgggtcgatgtttgatgttatggagcagcaacgatgttacgcagcagggcagtcgccctaaaacaaagttaaacatcatgagggaagcggtgatcgccgaagtatcgactcaactatcagaggtagttggcgtcatcgagcgccatctcgaaccgacgttgctggccgtacatttgtacggctccgcagtggatggcggcctgaagccacacagtgatattgatttgctggttacggtgaccgtaaggcttgatgaaacaacgcggcgagctttgatcaacgaccttttggaaacttcggcttcccctggagagagcgagattctccgcgctgtagaagtcaccattgttgtgcacgacgacatcattccgtggcgttatccagctaagcgcgaactgcaatttggagaatggcagcgcaatgacattcttgcaggtatcttcgagccagccacgatcgacattgatctggctatcttgctgacaaaagcaagagaacatagcgttgccttggtaggtccagcggcggaggaactctttgatccggttcctgaacaggatctatttgaggcgctaaatgaaaccttaacgctatggaactcgccgcccgactgggctggcgatgagcgaaatgtagtgcttacgttgtcccgcatttggtacagcgcagtaaccggcaaaatcgcgccgaaggatgtcgctgccgactgggcaatggagcgcctgccggcccagtatcagcccgtcatacttgaagctagacaggcttatcttggacaagaagaagatcgcttggcctcgcgcgcagatcagttggaagaatttgtccactacgtgaaaggcgagatcaccaaggtagtcggcaaataatgtctaacaattcgttcaagccgacgccgcttcgcggcgcggcttaactcaagcgttagatgcactaagcacataattgctcacagccaaactatcaggtcaagtctgcttttattatttttaagcgtgcataataagccctacacaaattgggagatatatcatgaaaggctggctttttcttgttatcgcaatagttggcgaagtaatcgcaacatagcttgcttggtcgttccgcgtgaacgtcggctcgattgtacctgcgttcaaatactttgcgatcgtgttgcgcgcctgcccggtgcgtcggctgatctcacggatcgactgcttctctcgcaacgccatccgacggatgatgtttaaaagtcccatgtggatcactccgttgccccgtcgctcaccgtgttggggggaaggtgcacatggctcagttctcaatggaaattatctgcctaaccggctcagttctgcgtagaaaccaacatgcaagctccaccgggtgcaaagcggcagcggcggcaggatatattcaattgtaaatggcttcatgtccgggaaatctacatggatcagcaatgagtatgatggtcaatatggagaaaaagaaagagtaattaccaattttttttcaattcaaaaatgtagatgtccgcagcgttattataaaatgaaagtacattttgataaaacgacaaattacgatccgtcgtatttataggcgaaagcaataaacaaattattctaattcggaaatctttatttcgacgtgtctacattcacgtccaaatgggggcttagatgagaaacttcacgatcggctctagttcgagcgatctagtaacatagatgacaccgcgcgcgataatttatcctagtttgcgcgctatattttgttttctatcgcgtattaaatgtataattgcgggactctaatcataaaaacccatctcataaataacgtcatgcattacatgttaattattacatgcttaacgtaattcaacagaaattatatgataatcatcgcaagaccggcaacaggattcaatcttaagaaactttattgccaaatgtttgaacgatcggggaaattcgtttctatgcttcaattctgctctatagatgttcttctagtcttaacttttagaaggcacaacatttgaaatgttggtaatttttctgctgggtagtgaaccattgtaatttgtgtttgcttatattatccgttgggtttctctatgttatctgtggggccatatcccagaactggttgagtcggtccaacacctgggtgccaatcatgtcgatggtggggtatggt

SEQ ID NO: 15 - DNA, 12734 bp, Artificial Sequence
  IPR252-pS-01
ccggattgaaagaaatatagtttaaatatttattgataaaataacaagtcaggtattatagtccaagcaaaaacataaatttattgatgcaagtttaaattcagaaatatttcaataactgattatatcagctggtacattgccgtagatgaaagactgagtgcgatattatgtgtaatacataaattgatgatatagctagcttagctcatcgggtcagaagaactcgtcaagaaggcgatagaaggcgatgcgctgcgaatcgggagcggcgataccgtaaagcacgaggaagcggtcagcccattcgccgccaagctcttcagcaatatcacgggtagccaacgctatgtcctgatagcggtccgccacacccagccggccacagtcgatgaatccagaaaagcggccattttccaccatgatattcggcaagcaggcatcgccatgagtcacgacgagatcctcgccgtcgggcatgcgcgccttgagcctggcgaacagttcggctggcgcgagcccctgatgctcttcgtccagatcatcctgatcgacaagaccggcttccatccgagtacgtgctcgctcgatgcgatgtttcgcttggtggtcgaatgggcaggtagccggatcaagcgtatgcagccgccgcattgcatcagccatgatggatactttctcggcaggagcaaggtgagatgacaggagatcctgccccggcacttcgcccaatagcagccagtcccttcccgcttcagtgacaacgtcgagcacagctgcgcaaggaacgcccgtcgtggccagccacgatagccgcgctgcctcgtcctgaagttcattcagggcaccggacaggtcggtcttgacaaaaagaaccgggcgcccctgcgctgacagccggaacacggcggcatcagagcagccgattgtctgttgtgcccagtcatagccgaatagcctctccacccaagcggccggagaacctgcgtgcaatccatcttgttcaatccaagctcccattttctgtgattttggatgtgtttttgtatggattgagagtgaatatgagactctaattggataccgaggggaatttatggaacgtcagtggagcatttttgacaagaaatatttgctagctgatagtgaccttaggcgacttttgaacgcgcaataatggtttctgacgtatgtgcttagctcattaaactccagaaacccgcggctgagtggctccttcaacgttgcggttctgtcagttccaaacgtaaaacggcttgtcccgcgtcatcggcgggggtcattccggactgtggggccatatcccagaactggttgagtcggtccaacacctgggtgccaatcatgtcgatggtggggtatggccaattttttttcaattcaaaaatgtagatgtccgcagcgttattataaaatgaaagtacattttgataaaacgacaaattacgatccgtcgtatttataggcgaaagcaataaacaaattattctaattcggaaatctttatttcgacgtgtctacattcacgtccaaatgggggcttagatgagaaacttcacgatcggctctagaggccatggcggccggaagacaaagatagcccggggcctgcaggaccaatgcattggatctggagacccgccggcggcagaagagatccaacaaaacattcacaatggattatagaaacatttgtttattcattataatgagatcttacattcatttaatattagaaaaagccacaaattcataacacaacaagccaagaaaaaaacacaaacttaagcacacaagctttttatttgacacaccaaatatttcatcttcatcttcatatgagctcgtcgacggtaccccctcaattagttacatcaccactttgtacaagaaagctgggtacaaatgtttgaacgatcggggaaattcgagctcggtaccgggccccccctcgagtttttttttttttttttttttagtctgaaaatttatccaactaatggaaactaaaaataagtcttaagaaattaaccaagaaaaagaaaaagagaaagaaaaaaacataatcaaagtatcacactgttcaccagcacacaacaacgcatataactaaagatctttaactattttttctaattgtcgttccaaactgtaaatgttggagcaacttctccaccaccttccccatggtaatacatattagagccaacattattcgtcattgccgcgggaaaatctccacctggcgactgctgggtctgctgctgctgagcaaagtaataatggtttcttgcgttataatcaaactcactagcagcgtaggcatcgcagttaaccggggctgcaaatccttgataaccaccataaccaacaacatttccacaaacagtaaccgaatcatccgaaacagaactttgatgatcgatattagtcatgaggctctgcgtgttgctcaagaaatggtgttgatcatcctcttgtttgaaacaagccctagcactctccgaagacaagtttcctccattgtaataataaccattgtacctctcttgatgttggtgcaataagctcaaatctactccctgatgatgctgaaccgcagcgttttgccaaccgctagcactattctcactctctgaaacgttattactgatcatcatcatacttggaaccggacggttagcctccttgagacgttttgcggcgctaccaataggaagactagggctttcgaggattgctttaacgttgtatctgttcatgtcgaagttagtcactgcggttaatcctctgaatttgatggccgcaatgtcgtatgcctctgcagcttcttcttgtgtgccaaaagttcccaagtagaggtctttgttaccggcgactcttcctatcctagcttgccatcttccatgttggtgatgtcttgttactccacgataaatcgatgcaccacgagagaaaccactacttttcctgcgcagtgaggcaacatactcttgccttgtcatgtgcttcatctcttctacctctttttcatattcgctcatggggaagttagtagtagtggtggttccccaatacttgagtgcggctaaatcataagccctagctgctttttcttctttgtcataacctcccaaataaacttgtcttcctttgcgcgtttggccttctcttttacaactattatcccataaatgtgcctcatatcttcctgtccaccgatgccttgtaacaccgcggtatatagacgtcctctgtccaaaactctcaatagttttcttcggtgtagcttcaacgctatcatcaatagtcttcccttgggcaacaacgttgttattgctgtcgttgttgttatcacaagaagtagatgagttcattgagagggacaggccttttgcagcattgccattttcttgattatcaacattatccacgggttgatttctcagccatgtctttatcatcgaaagtcctagtgagccaccaccaccgtctcctcctccataacagccacttccacttccatctccaacgttttcgttggtgttgtaaatcgtggtggtgcggccaaggaaattctcaagctttggtccatcttgctcatcgttgtggatgttattgcatgcacaaccattgatgtcccaatctcgggagtgactattgttgtctctggtgaaagcatcgacgacgacaccaaagggagaaggaaacgatgtttggatggctgaagactcatcggaggcagcggtcggatcgtaacagtactctccggcgacatctacgacggttgtggtggtggaagagtagacgtccttacgatggtgattttgttcataaggagagagagaaaagcctaaccagttattatccattgagcctgcttttttgtacaaacttgtgatcgggatctgtaattgtaatgttgtttgttgtttgttgttgttggtaattgtggatcctctagagtcccccgtgtcctctccaaatgaaatgaacttccttatatagaggaagggtcttgcgaaggatagtgggattgtgcgtcatcccttacgtcagtggagatatcacatcaatccacttgctttgaagacgtggttggaacgtcttctttttccacgatgctcctcgtgggtgggggtccatctttgggaccactgtcggcagaggcatcttcaacgatggcctttcctttatcgcaatgatggcatttgtaggagccaccttccttttccactatcttcacaataaagtgacagatagctgggcaatggaatccgaggaggtttccggatattaccctttgttgaaaagtctcaattgccctttggtcttctgagactgtatctttgatatttttggagtagacaagtgtgtcgtgctccaccatgttgacgaagattttcttcttgtcattgagtcgtaagagactctgtatgaactgttcgccagtctttacggcgagttctgttaggtcctctatttgaatctttgactccatggcctttgattcagtgggaactacctttttagagactccaatctctattacttgcctcgccggcgggtctcgggatcccctgcaggactagtggatttgtcttcaaggccttaagggccagatcttgggcccggtacccgatcagattgtcgtttcccgccttcggtttaaactatcagtgtttgacaggatatattggcgggtaaacctaagagaaaagagcgtttattagaataatcggatatttaaaagggcgtgaaaaggtttatccgttcgtccatttgtatgtgcatgccaaccacagggttcccctcgggagtgcttggcattccgtgcgataatgacttctgttcaaccacccaaacgtcggaaagcctgacgacggagcagcattccaaaaagatcccttggctcgtctgggtcggctagaaggtcgagtgggctgctgtggcttgatccctcaacgcggtcgcggacgtagcgcagcgccgaaaaatcctcgatcgcaaatccgacgctgtcgaaaagcgtgatctgcttgtcgctctttcggccgacgtcctggccagtcatcacgcgccaaagttccgtcacaggatgatctggcgcgagttgctggatctcgccttcaatccgggtctgtggcgggaactccacgaaaatatccgaacgcagcaagatatcgcggtgcatctcggtcttgcctgggcagtcgccgccgacgccgttgatgtggacgccgaaaaggatctaggtgaagatcctttttgataatctcatgaccaaaatcccttaacgtgagttttcgttccactgagcgtcagaccccgtagaaaagatcaaaggatcttcttgagatcctttttttctgcgcgtaatctgctgcttgcaaacaaaaaaaccaccgctaccagcggtggtttgtttgccggatcaagagctaccaactctttttccgaaggtaactggcttcagcagagcgcagataccaaatactgttcttctagtgtagccgtagttaggccaccacttcaagaactctgtagcaccgcctacatacctcgctctgctaatcctgttaccagtggctgctgccagtggcgataagtcgtgtcttaccgggttggactcaagacgatagttaccggataaggcgcagcggtcgggctgaacggggggttcgtgcacacagcccagcttggagcgaacgacctacaccgaactgagatacctacagcgtgagctatgagaaagcgccacgcttcccgaagggagaaaggcggacaggtatccggtaagcggcagggtcggaacaggagagcgcacgagggagcttccagggggaaacgcctggtatctttatagtcctgtcgggtttcgccacctctgacttgagcgtcgatttttgtgatgctcgtcaggggggcggagcctatggaaaaacgccagcaacgcggcctttttacggttcctggccttttgctggccttttgctcacatgttctttcctgcgttatcccctgattctgtggataaccgattaccgcctttgagtgagctgataccgctcgccgcagccgaacgaccgagcgcagcgagtcagtgagcgaggaagcggaagagcgcctgatgcggtattttctccttacgcatctgtgcggtatttcacaccgcatatggtgcactctcagtacaatctgctctgatgccgcatagttaagccagtatacactccgctatcgctacgtgactgggtcatggctgcgccccgacacccgccaacacccgctgacgcgccctgacgggcttgtctgctcccggcatccgcttacagacaagctgtgaccgtctccgggagctgcatgtgtcagaggttttcaccgtcatcaccgaaacgcgcgaggcaggggtacgtcgaggtcgatccaacccctccgctgctatagtgcagtcggcttctgacgttcagtgcagccgtcttctgaaaacgacatgtcgcacaagtcctaagttacgcgacaggctgccgccctgcccttttcctggcgttttcttgtcgcgtgttttagtcgcataaagtagaatacttgcgactagaaccggagacattacgccatgaacaagagcgccgccgctggcctgctgggctatgcccgcgtcagcaccgacgaccaggacttgaccaaccaacgggccgaactgcacgcggccggctgcaccaagctgttttccgagaagatcaccggcaccaggcgcgaccgcccggagctggccaggatgcttgaccacctacgccctggcgacgttgtgacagtgaccaggctagaccgcctggcccgcagcacccgcgacctactggacattgccgagcacatccaggaggccggcgcgggcctgcgtagcctggcagagccgtgggccgacaccaccacgccggccggccgcatggtgttgaccgtgttcgccggcattgccgagttcgagcgttccctaatcatcgaccgcacccggagcgggcgcgaggccgccaaggcgcgaggcgtgaagtttggcccccgccctaccctcaccccggcacagatcgcgcacgcccgcgagctgatcgaccaggaaggccgcaccgtgaaagaggcggctgcactgcttggcgtgcatcgctcgaccctgtaccgcgcacttgagcgcagcgaggaagtgacgcccaccgaggccaggcggcgcggtgccttccgtgaggacgcattgaccgaggccgacgccctggcggccgccgagaatgaacgccaagaggaacaagcatgaaaccgcaccaggacggccaggacgaaccgtttttcattaccgaagagatcgaggcggagatgatcgcggccgggtacgtgttcgagccgcccgcgcacgtctcaaccgtgcggctgcatgaaatcctggccggtttgtctgatgccaagctcgcggcctggccggcgagcttggccgctgaagaaaccgagcgccgccgtctaaaaaggtgatgtgtatttgagtaaaacagcttgcgtcatgcggtcgctgcgtatatgatgcgatgagtaaataaacaaatacgcaaggggaacgcatgaaggttatcgctgtacttaaccagaaaggcgggtcaggcaagacgaccatcgcaacccatctagcccgcgccctgcaactcgccggggccgatgttctgttagtcgattccgatccccagggcagtgcccgcgattgggcggccgtgcgggaagatcaaccgctaaccgttgtcggcatcgaccgcccgacgattgaccgcgacgtgaaggccatcggccggcgcgacttcgtagtgatcgacggagcgccccaggcggcggacttggctgtgtccgcgatcaaggcagccgacttcgtgctgattccggtgcagccaagcccttacgacatatgggccaccgccgacctggtggagctggttaagcagcgcattgaggtcacggatggaaggctacaagcggcctttgtcgtgtcgcgggcgatcaaaggcacgcgcatcggcggtgaggttgccgaggcgctggccgggtacgagctgcccattcttgagtcccgtatcacgcagcgcgtgagctacccaggcactgccgccgccggcacaaccgttcttgaatcagaacccgagggcgacgctgcccgcgaggtccaggcgctggccgctgaaattaaatcaaaactcatttgagttaatgaggtaaagagaaaatgagcaaaagcacaaacacgctaagtgccggccgtccgagcgcacgcagcagcaaggctgcaacgttggccagcctggcagacacgccagccatgaagcgggtcaactttcagttgccggcggaggatcacaccaagctgaagatgtacgcggtacgccaaggcaagaccattaccgagctgctatctgaatacatcgcgcagctaccagagtaaatgagcaaatgaataaatgagtagatgaattttagcggctaaaggaggcggcatggaaaatcaagaacaaccaggcaccgacgccgtggaatgccccatgtgtggaggaacgggcggttggccaggcgtaagcggctgggttgtctgccggccctgcaatggcactggaacccccaagcccgaggaatcggcgtgagcggtcgcaaaccatccggcccggtacaaatcggcgcggcgctgggtgatgacctggtggagaagttgaaggcggcgcaggccgcccagcggcaacgcatcgaggcagaagcacgccccggtgaatcgtggcaagcggccgctgatcgaatccgcaaagaatcccggcaaccgccggcagccggtgcgccgtcgattaggaagccgcccaagggcgacgagcaaccagattttttcgttccgatgctctatgacgtgggcacccgcgatagtcgcagcatcatggacgtggccgttttccgtctgtcgaagcgtgaccgacgagctggcgaggtgatccgctacgagcttccagacgggcacgtagaggtttccgcagggccggccggcatggcgagtgtgtgggattacgacctggtactgatggcggtttcccatctaaccgaatccatgaaccgataccgggaagggaagggagacaagcccggccgcgtgttccgtccacacgttgcggacgtactcaagttctgccggcgagccgatggcggaaagcagaaagacgacctggtagaaacctgcattcggttaaacaccacgcacgttgccatgcagcgtacgaagaaggccaagaacggccgcctggtgacggtatccgagggtgaagccttgattagccgctacaagatcgtaaagagcgaaaccgggcggccggagtacatcgagatcgagctagctgattggatgtaccgcgagatcacagaaggcaagaacccggacgtgctgacggttcaccccgattactttttgatcgatcccggcatcggccgttttctctaccgcctggcacgccgcgccgcaggcaaggcagaagccagatggttgttcaagacgatctacgaacgcagtggcagcgccggagagttcaagaagttctgtttcaccgtgcgcaagctgatcgggtcaaatgacctgccggagtacgatttgaaggaggaggcggggcaggctggcccgatcctagtcatgcgctaccgcaacctgatcgaaggcgaagcatccgccggttcctaatgtacggagcagatgctagggcaaattgccctagcaggggaaaaaggtcgaaaaggtctctttcctgtggatagcacgtacattgggaacccaaagccgtacattgggaaccggaacccgtacattgggaacccaaagccgtacattgggaaccggtcacacatgtaagtgactgatataaaagagaaaaaaggcgatttttccgcctaaaactctttaaaacttattaaaactcttaaaacccgcctggcctgtgcataactgtctggccagcgcacagccgaagagctgcaaaaagcgcctacccttcggtcgctgcgctccctacgccccgccgcttcgcgtcggcctatcgcggccgctggccgctcaaaaatggctggcctacggccaggcaatctaccagggcgcggacaagccgcgccgtcgccactcgaccgccggcgcccacatcaaggcaccggtgggtatgcctgacgatgcgtggagaccgaaaccttgcgctcgttcgccagccaggacagaaatgcctcgacttcgctgctgcccaaggttgccgggtgacgcacaccgtggaaacggatgaaggcacgaacccagtggacataagcctgttcggttcgtaagctgtaatgcaagtagcgtatgcgctcacgcaactggtccagaaccttgaccgaacgcagcggtggtaacggcgcagtggcggttttcatggcttgttatgactgtttttttggggtacagtctatgcctcgggcatccaagcagcaagcgcgttacgccgtgggtcgatgtttgatgttatggagcagcaacgatgttacgcagcagggcagtcgccctaaaacaaagttaaacatcatgagggaagcggtgatcgccgaagtatcgactcaactatcagaggtagttggcgtcatcgagcgccatctcgaaccgacgttgctggccgtacatttgtacggctccgcagtggatggcggcctgaagccacacagtgatattgatttgctggttacggtgaccgtaaggcttgatgaaacaacgcggcgagctttgatcaacgaccttttggaaacttcggcttcccctggagagagcgagattctccgcgctgtagaagtcaccattgttgtgcacgacgacatcattccgtggcgttatccagctaagcgcgaactgcaatttggagaatggcagcgcaatgacattcttgcaggtatcttcgagccagccacgatcgacattgatctggctatcttgctgacaaaagcaagagaacatagcgttgccttggtaggtccagcggcggaggaactctttgatccggttcctgaacaggatctatttgaggcgctaaatgaaaccttaacgctatggaactcgccgcccgactgggctggcgatgagcgaaatgtagtgcttacgttgtcccgcatttggtacagcgcagtaaccggcaaaatcgcgccgaaggatgtcgctgccgactgggcaatggagcgcctgccggcccagtatcagcccgtcatacttgaagctagacaggcttatcttggacaagaagaagatcgcttggcctcgcgcgcagatcagttggaagaatttgtccactacgtgaaaggcgagatcaccaaggtagtcggcaaataatgtctaacaattcgttcaagccgacgccgcttcgcggcgcggcttaactcaagcgttagatgcactaagcacataattgctcacagccaaactatcaggtcaagtctgcttttattatttttaagcgtgcataataagccctacacaaattgggagatatatcatgaaaggctggctttttcttgttatcgcaatagttggcgaagtaatcgcaacatagcttgcttggtcgttccgcgtgaacgtcggctcgattgtacctgcgttcaaatactttgcgatcgtgttgcgcgcctgcccggtgcgtcggctgatctcacggatcgactgcttctctcgcaacgccatccgacggatgatgtttaaaagtcccatgtggatcactccgttgccccgtcgctcaccgtgttggggggaaggtgcacatggctcagttctcaatggaaattatctgcctaaccggctcagttctgcgtagaaaccaacatgcaagctccaccgggtgcaaagcggcagcggcggcaggatatattcaattgtaaatggcttcatgtccgggaaatctacatggatcagcaatgagtatgatggtcaatatggagaaaaagaaagagtaattaccaattttttttcaattcaaaaatgtagatgtccgcagcgttattataaaatgaaagtacattttgataaaacgacaaattacgatccgtcgtatttataggcgaaagcaataaacaaattattctaattcggaaatctttatttcgacgtgtctacattcacgtccaaatgggggcttagatgagaaacttcacgatcggctctagttcgagcgatctagtaacatagatgacaccgcgcgcgataatttatcctagtttgcgcgctatattttgttttctatcgcgtattaaatgtataattgcgggactctaatcataaaaacccatctcataaataacgtcatgcattacatgttaattattacatgcttaacgtaattcaacagaaattatatgataatcatcgcaagaccggcaacaggattcaatcttaagaaactttattgccaaatgtttgaacgatcggggaaattcgtttctatgcttcaattctgctctatagatgttcttctagtcttaacttttagaaggcacaacatttgaaatgttggtaatttttctgctgggtagtgaaccattgtaatttgtgtttgcttatattatccgttgggtttctctatgttatctgtggggccatatcccagaactggttgagtcggtccaacacctgggtgccaatcatgtcgatggtggggtatggt

SEQ ID NO: 16 - DNA, 5472 bp, Artificial Sequence
  IPR 252-pK-02
cggacgaccctgcgcgctcagacgaaacaccgccgcatcagagcagccaatggtctgctgcgcccaatcatagccaaacagacgttccacccacgctgccgggctacccgcatgcaggccatcctgttcaatcatactcttcctttttcaatattattgaagcatttatcagggttattgtctcatgagcggatacatatttgaatgtatttagaaaaataaacaaataggggttccgcgcacatttccccgaaaagtgccacctaaattgtaagcgttaatattttgttaaaattcgcgttaaatttttgttaaatcagctcattttttaaccaataggccgaaatcggcaaaatcccttataaatcaaaagaatagaccgagatagggttgagtggccgctacagggcgctcccattcgccattcaggctgcgcaactgttgggaagggcgtttcggtgcgggcctcttcgctattacgccagctggcacgacaggtttcccgactggaaagcgggcagtgagcgcaacgcaattaatgtgagttagctcactcattaggcaccccaggctttacactttatgcttccggctcgtatgttgtgtggaattgtgagcggataacaatttcacacaggaaacagctatgaccatgattacgccaagctcgaaattaaccctcactaaagggaacaaaagctggactagaggcccttaaggccttgaagacaaatccactagtcctgcaggggatcccgagacccgccggcgaggcaagtaatagagattggagtctctaaaaaggtagttcccactgaatcaaaggccatggagtcaaagattcaaatagaggacctaacagaactcgccgtaaagactggcgaacagttcatacagagtctcttacgactcaatgacaagaagaaaatcttcgtcaacatggtggagcacgacacacttgtctactccaaaaatatcaaagatacagtctcagaagaccaaagggcaattgagacttttcaacaaagggtaatatccggaaacctcctcggattccattgcccagctatctgtcactttattgtgaagatagtggaaaaggaaggtggctcctacaaatgccatcattgcgataaaggaaaggccatcgttgaagatgcctctgccgacagtggtcccaaagatggacccccacccacgaggagcatcgtggaaaaagaagacgttccaaccacgtcttcaaagcaagtggattgatgtgatatctccactgacgtaagggatgacgcacaatcccactatccttcgcaagacccttcctctatataaggaagttcatttcatttggagaggacacgggggactctagaggatccacaattaccaacaacaacaaacaacaaacaacattacaattacagatcccgatcacaagtttgtacaaaaaagcaggctcaatggataataactggttaggcttttctctctctccttatgaacaaaatcaccatcgtaaggacgtctactcttccaccaccacaaccgtcgtagatgtcgccggagagtactgttacgatccgaccgctgcctccgatgagtcttcagccatccaaacatcgtttccttctccctttggtgtcgtcgtcgatgctttcaccagagacaacaatagtcactcccgagattgggacatcaatggttgtgcatgcaataacatccacaacgatgagcaagatggaccaaagcttgagaatttccttggccgcaccaccacgatttacaacaccaacgaaaacgttggagatggaagtggaagtggctgttatggaggaggagacggtggtggtggctcactaggactttcgatgataaagacatggctgagaaatcaacccgtggataatgttgataatcaagaaaatggcaatgctgcaaaaggcctgtccctctcaatgaactcatctacttcttgtgataacaacaacgacagcaataacaacgttgttgcccaagggaagactattgatgatagcgttgaagctacaccgaagaaaactattgagagttttggacagaggacgtctatataccgcggtgttacaaggcatcggtggacaggaagatatgaggcacatttatgggataatagttgtaaaagagaaggccaaacgcgcaaaggaagacaagtttatttgggaggttatgacaaagaagaaaaagcagctagggcttatgatttagccgcactcaagtattggggaaccaccactactactaacttccccatgagcgaatatgaaaaagaggtagaagagatgaagcacatgacaaggcaagagtatgttgcctcactgcgcaggaaaagtagtggtttctctcgtggtgcatcgatttatcgtggagtaacaagacatcaccaacatggaagatggcaagctaggataggaagagtcgccggtaacaaagacctctacttgggaacttttggcacacaagaagaagctgcagaggcatacgacattgcggccatcaaattcagaggattaaccgcagtgactaacttcgacatgaacagatacaacgttaaagcaatcctcgaaagccctagtcttcctattggtagcgccgcaaaacgtctcaaggaggctaaccgtccggttccaagtatgatgatgatcagtaataacgtttcagagagtgagaatagtgctagcggttggcaaaacgctgcggttcagcatcatcagggagtagatttgagcttattgcaccaacatcaagagaggtacaatggttattattacaatggaggaaacttgtcttcggagagtgctagggcttgtttcaaacaagaggatgatcaacaccatttcttgagcaacacgcagagcctcatgactaatatcgatcatcaaagttctgtttcggatgattcggttactgtttgtggaaatgttgttggttatggtggttatcaaggatttgcagccccggttaactgcgatgcctacgctgctagtgagtttgattataacgcaagaaaccattattactttgctcagcagcagcagacccagcagtcgccaggtggagattttcccgcggcaatgacgaataatgttggctctaatatgtattaccatggggaaggtggtggagaagttgctccaacatttacagtttggaacgacaattagaaaaaatagttaaagatctttagttatatgcgttgttgtgtgctggtgaacagtgtgatactttgattatgtttttttctttctctttttctttttcttggttaatttcttaagacttatttttagtttccattagttggataaattttcagactaaaaaaaaaaaaaaaaaaaaactcgagggggggcccggtaccgagctcgaatttccccgatcgttcaaacatttgtacccagctttcttgtacaaagtggtgatgtaactaattgagggggtaccgtcgacgagctcatatgaagatgaagatgaaatatttggtgtgtcaaataaaaagcttgtgtgcttaagtttgtgtttttttcttggcttgttgtgttatgaatttgtggctttttctaatattaaatgaatgtaagatctcattataatgaataaacaaatgtttctataatccattgtgaatgttttgttggatctcttctgccgccggcgggtctccagatccaatgcattggtcctgcaggccccgggctatctttgtcttccggccgccatggccagatcgtacccaattcgccctatagtgagtcgtattacaattcactggccgtcgttttacaacgtcgtgactgggaaaaccctggcgttacccaacttaatcgccttgcagcacatccccctttcgccagctgcattaacatggtcatagctgtttccttgcgtattgggcgctctccgcttcctcgctcactgactcgctgcgctcggtcgttcgggtaaagcctggggtgcctaatgagcaaaaggccagcaaaaggccaggaaccgtaaaaaggccgcgttgctggcgtttttccataggctccgcccccctgacgagcatcacaaaaatcgacgctcaagtcagaggtggcgaaacccgacaggactataaagataccaggcgtttccccctggaagctccctcgtgcgctctcctgttccgaccctgccgcttaccggatacctgtccgcctttctcccttcgggaagcgtggcgctttctcatagctcacgctgtaggtatctcagttcggtgtaggtcgttcgctccaagctgggctgtgtgcacgaaccccccgttcagcccgaccgctgcgccttatccggtaactatcgtcttgagtccaacccggtaagacacgacttatcgccactggcagcagccactggtaacaggattagcagagcgaggtatgtaggcggtgctacagagttcttgaagtggtggcctaactacggctacactagaagaacagtatttggtatctgcgctctgctgaagccagttaccttcggaaaaagagttggtagctcttgatccggcaaacaaaccaccgctggtagcggtggtttttttgtttgcaagcagcagattacgcgcagaaaaaaaggatctcaagaagatcctttgatcttttctacggggtctgacgctcagtggaacgaaaactcacgttaagggattttggtcatgagattatcaaaaaggatcttcacctagatccttttaaattaaaaatgaagttttaaatcaatctaaagtatatatgagtaaacttggtctgacagttattagaaaaattcatccagcagacgataaaacgcaatacgctggctatccggtgccgcaatgccatacagcaccagaaaacgatccgcccattcgccgcccagttcttccgcaatatcacgggtggccagcgcaatatcctgataacgatccgccacgcccagacggccgcaatcaataaagccgctaaaacggccattttccaccataatgttcggcaggcacgcatcaccatgggtcaccaccagatcttcgccatccggcatgctcgctttcagacgcgcaaacagctctgccggtgccaggccctgatgttcttcatccagatcatcctgatccaccaggcccgcttccatacgggtacgcgcacgttcaatacgatgtttcgcctgatgatcaaacggacaggtcgccgggtccagggtatgcagacgacgcatggcatccgccataatgctcactttttctgccggcgccagatggctagacagcagatcctgacccggcacttcgcccagcagcagccaatcacggcccgcttcggtcaccacatccagcaccgccgcacacggaacaccggtggtggccagccagctcagacgcgccgcttcatcctgcagctcgttcagcgcaccgctcagatcggttttcacaaacagcac

SEQ ID NO: 17 - DNA, 11632 bp, Artificial Sequence; identical to SEQ ID NO: 5
  vector pZFN-nptII-70s::TDT